European Patent Application EP 4 115 737 A1, published January 11, 2023. Title: BVP8 PROTEIN FOR KILLING TETRANYCHID MITES AND USE THEREOF. Applicant: Hubei Biopesticide Engineering Research Center. The sequence listing filed with the application follows.

SEQUENCE LISTING (2 sequences)

SEQ ID NO: 1 - DNA, 231 bp, Artificial Sequence
ttgttcggaccaattttaaaagcattaaaagctcttgtatctaaagtaccgtggggtaaggtcgcatcattcttaaaatgggcaggtaacttagctgctgcagccgctaaatattcatatacaagtggaaagaaaatccttgcgtatatccaaaaacacccaggaaaaatcgttgattggttcctaaaaggatattctgtatacgacgttattaaaatgattcttggctaa

SEQ ID NO: 2 - protein, 70 aa, Artificial Sequence
MFGPILKALKALVSKVPWGKVASFLKWAGNLAAAAAKYSYTSGKKILAYIQKHPGKIVDWFLKGYSVYDV